European Patent Application EP 4 306 545 A1, published January 17, 2024. Title: FUSION PROTEIN OF TNFR2 AND APRIL BAFF RECEPTOR. Applicant: SHANGHAI CELGEN BIO-PHARMACEUTICAL CO., LTD. The sequence listing filed with the application follows.

SEQUENCE LISTING (20 sequences)

SEQ ID NO: 1 - protein, 18 aa, Artificial Sequence
  primer KDP068
CTTTGGCAAAGAATTGGG

SEQ ID NO: 2 - protein, 20 aa, Artificial Sequence
  primer KDP422
GTCGCCAGTGCTCCCTTCAG

SEQ ID NO: 3 - protein, 39 aa, Artificial Sequence
  primer KDP410
CTGAAGGGAGCACTGGCGACGGGCAGTGCTCCCAAAATG

SEQ ID NO: 4 - protein, 39 aa, Artificial Sequence
  primer KDP411
TATCACAGCTCTTGGGCTCCGCATTCGTTCCTTTCACTG

SEQ ID NO: 5 - protein, 19 aa, Artificial Sequence
  primer KDP134
GAGCCCAAGAGCTGTGATA

SEQ ID NO: 6 - protein, 22 aa, Artificial Sequence
  primer BGHR
AACTAGAAGGCACAGTCGAGGC

SEQ ID NO: 7 - protein, 19 aa, Artificial Sequence
  primer KDP066
CGAACATCGATTGAATTCC

SEQ ID NO: 8 - protein, 19 aa, Artificial Sequence
  primer KDP093
TCTAGCATTTAGGTGACAC

SEQ ID NO: 9 - protein, 39 aa, Artificial Sequence
  primer KDP408
CTGAAGGGAGCACTGGCGACGACGCGCCAGCCCCCACGC

SEQ ID NO: 10 - protein, 37 aa, Artificial Sequence
  primer KDP409
TATCACAGCTCTTGGGCTCGGCCGGTTTCGGCCGCGG

SEQ ID NO: 11 - protein, 41 aa, Artificial Sequence
  primer KDP412
CTGAAGGGAGCACTGGCGACTCACTCAGCTGCCGCAAGGAG

SEQ ID NO: 12 - protein, 41 aa, Artificial Sequence
  primer KDP413
TATCACAGCTCTTGGGCTCCCTGAGCTTGTTCTCACAGAAG

SEQ ID NO: 13 - protein, 235 aa, Artificial Sequence
  TNFR2 amino acid sequence
LPAQVAFTPYAPEPGSTCRLREYYDQTAQMCCSKCSPGQHAKVFCTKTSDTVCDSCEDSTYTQLWNWVPECLSCGSRCSSDQVETQACTREQNRICTCRPGWYCALSKQEGCRLCAPLRKCRPGFGVARPGTETSDVVCKPCAPGTFSNTTSSTDICRPHQICNVVAIPGNASMDAVCTSTSPTRSMAPGAVHLPQPVSTRSQHTQPTPEPSTAPSTSFLLPMGPSPPAEGSTGD

SEQ ID NO: 14 - protein, 293 aa, Artificial Sequence
  TACI amino acid sequence
MSGLGRSRRGGRSRVDQEERFPQGLWTGVAMRSCPEEQYWDPLLGTCMSCKTICNHQSQRTCAAFCRSLSCRKEQGKFYDHLLRDCISCASICGQHPKQCAYFCENKLRSPVNLPPELRRQRSGEVENNSDNSGRYQGLEHRGSEASPALPGLKLSADQVALVYSTLGLCLCAVLCCFLVAVACFLKKRGDPCSCQPRSRPRQSPAKSSQDHAMEAGSPVSTSPEPVETCSFCFPECRAPTQESAVTPGTPDPTCAGRWGCHTRTTVLQPCPHIPDSGLGIVCVPAQEGGPGA

SEQ ID NO: 15 - protein, 184 aa, Artificial Sequence [sequence omitted]

SEQ ID NO: 16 - protein, 184 aa, Artificial Sequence
  BAFFR amino acid sequence
MRRGPRSLRGRDAPAPTPCVPAECFDLLVRHCVACGLLRTPRPKPAGASSPAPRTALQPQESVGAGAGEAALPLPGLLFGAPALLGLALVLALVLVGLVSWRRRQRRLRGASSAEAPDGDKDAPEPLDKVIILSPGISDATAPAWPPPGEDPGTTPPGHSVPVPATELGSTELVTTKTAGPEQQ

SEQ ID NO: 17 - protein, 231 aa, Artificial Sequence
  amino acid sequence of Fc fragment
EPKSCDKTHTCPPCPAPELLGGPSVFLFPPKPKDTLMISRTPEVTCVVVDVSHEDPEVKFNWYVDGVEVHNAKTKPREEQYNSTYRVVSVLTVLHQDWLNGKEYKCKVSNKALPAPIEKTISKAKGQPREPQVYTLPPSREEMTKNQVSLTCLVKGFYPSDIAVEWESNGQPENNYKTTPPVLDSDGSFFLYSKLTVDKSRWQQGNVFSCSVMHEALHNHYTQKSLSLSPG

SEQ ID NO: 18 - protein, 508 aa, Artificial Sequence
  amino acid sequence of TNFR2-TACI-Fc  fusion protein
LPAQVAFTPYAPEPGSTCRLREYYDQTAQMCCSKCSPGQHAKVFCTKTSDTVCDSCEDSTYTQLWNWVPECLSCGSRCSSDQVETQACTREQNRICTCRPGWYCALSKQEGCRLCAPLRKCRPGFGVARPGTETSDVVCKPCAPGTFSNTTSSTDICRPHQICNVVAIPGNASMDAVCTSTSPTRSMAPGAVHLPQPVSTRSQHTQPTPEPSTAPSTSFLLPMGPSPPAEGSTGDSLSCRKEQGKFYDHLLRDCISCASICGQHPKQCAYFCENKLREPKSCDKTHTCPPCPAPELLGGPSVFLFPPKPKDTLMISRTPEVTCVVVDVSHEDPEVKFNWYVDGVEVHNAKTKPREEQYNSTYRVVSVLTVLHQDWLNGKEYKCKVSNKALPAPIEKTISKAKGQPREPQVYTLPPSREEMTKNQVSLTCLVKGFYPSDIAVEWESNGQPENNYKTTPPVLDSDGSFFLYSKLTVDKSRWQQGNVFSCSVMHEALHNHYTQKSLSLSPG

SEQ ID NO: 19 - protein, 515 aa, Artificial Sequence
  amino acid sequence of TNFR2-BCMA-Fc
LPAQVAFTPYAPEPGSTCRLREYYDQTAQMCCSKCSPGQHAKVFCTKTSDTVCDSCEDSTYTQLWNWVPECLSCGSRCSSDQVETQACTREQNRICTCRPGWYCALSKQEGCRLCAPLRKCRPGFGVARPGTETSDVVCKPCAPGTFSNTTSSTDICRPHQICNVVAIPGNASMDAVCTSTSPTRSMAPGAVHLPQPVSTRSQHTQPTPEPSTAPSTSFLLPMGPSPPAEGSTGDGQCSQNEYFDSLLHACIPCQLRCSSNTPPLTCQRYCNASVTNSVKGTNAEPKSCDKTHTCPPCPAPELLGGPSVFLFPPKPKDTLMISRTPEVTCVVVDVSHEDPEVKFNWYVDGVEVHNAKTKPREEQYNSTYRVVSVLTVLHQDWLNGKEYKCKVSNKALPAPIEKTISKAKGQPREPQVYTLPPSREEMTKNQVSLTCLVKGFYPSDIAVEWESNGQPENNYKTTPPVLDSDGSFFLYSKLTVDKSRWQQGNVFSCSVMHEALHNHYTQKSLSLSPG

SEQ ID NO: 20 - protein, 501 aa, Artificial Sequence
  amino acid sequence of TNFR2-BAFFR-Fc
LPAQVAFTPYAPEPGSTCRLREYYDQTAQMCCSKCSPGQHAKVFCTKTSDTVCDSCEDSTYTQLWNWVPECLSCGSRCSSDQVETQACTREQNRICTCRPGWYCALSKQEGCRLCAPLRKCRPGFGVARPGTETSDVVCKPCAPGTFSNTTSSTDICRPHQICNVVAIPGNASMDAVCTSTSPTRSMAPGAVHLPQPVSTRSQHTQPTPEPSTAPSTSFLLPMGPSPPAEGSTGDDAPAPTPCVPAECFDLLVRHCVACGLLRTPRPKPAEPKSCDKTHTCPPCPAPELLGGPSVFLFPPKPKDTLMISRTPEVTCVVVDVSHEDPEVKFNWYVDGVEVHNAKTKPREEQYNSTYRVVSVLTVLHQDWLNGKEYKCKVSNKALPAPIEKTISKAKGQPREPQVYTLPPSREEMTKNQVSLTCLVKGFYPSDIAVEWESNGQPENNYKTTPPVLDSDGSFFLYSKLTVDKSRWQQGNVFSCSVMHEALHNHYTQKSLSLSPG